European Patent Specification EP 3 640 257 B1, published May 14, 2025. Title: Novel polypeptide and a method for producing putrescine using the same. Applicant: CJ CheilJedang Corporation. The sequence listing filed with the application follows.

SEQUENCE LISTING (68 sequences)

SEQ ID NO: 1 - protein, 494 aa, Artificial Sequence
  ATCC13032 NCgl2522
MTSETLQAQAPTKTQRWAFLAVISGGLFLIGVDNSILYTALPLLREQLAATETQALWIINAYPLLMAGLLLGTGTLGDKIGHRRMFLMGLSIFGIASLGAAFAPTAWALVAARAFLGIGAATMMPATLALIRITFEDERERNTAIGIWGSVAILGAAAGPIIGGALLEFFWWGSVFLINVPVAVIALIATLFVAPANIANPSKHWDFLSSFYALLTLAGLIITIKESVNTARHMPLLLGAVIMLIIGAVLFSSRQKKIEEPLLDLSLFRNRLFLGGVVAAGMAMFTVSGLEMTTSQRFQLSVGFTPLEAGLLMIPAALGSFPMSIIGGANLHRWGFKPLISGGFAATAVGIALCIWGATHTDGLPFFIAGLFFMGAGAGSVMSVSSTAIIGSAPVRKAGMASSIEEVSYEFGTLLSVAILGSLFPFFYSLHAPAEVADNFSAGVHHAIDGDAARASLDTAYINVLIIALVCAVAAALISSYLFRGNPKGANNAH

SEQ ID NO: 2 - protein, 494 aa, Artificial Sequence
  ATCC13869 NCgl2522
MISETLQAQAPTKTQRWAFLAVISGGLFLIGVDNSILYTALPLLREQLAATETQALWIINAYPLLMAGLLLGTGTLGDKIGHRRMFLMGLSIFGIASLGAAFAPTAWALVAARAFLGIGAATMMPATLALIRITFEDERERNTAIGIWGSVAILGAAAGPIIGGALLEFFWWGSVFLINVPVAVIALIATLFVAPANIANPSKHWDFLSSFYALLTLAGLIVTIKESVNTARHLPLLVGAIILLIIGAVLFSSRQKKIEEPLLDLSLFRNRLFLGGVVAAGMAMFTVSGLEMTTSQRFQLSVGFTPLEAGLLMIPAALGSFPMSIIGGANLHRWGFKPLISGGFLATAVGIALCIWGATHTDGLPFFIAGLFFMGAGAGSVMSVSSTAIIGSAPVRKAGMASSIEEVSYEFGTLLSVAILGSLFPFFYSLHAPAEVADNFSAGVHHAIYGDAARASLDTAYINVLIIALVCAVAAALISSYLFRGNPKGANNAH

SEQ ID NO: 3 - protein, 494 aa, Artificial Sequence
  ATCC13032 NCgl2522_M1
MTSETLQAQAPTKTQRWAFLAVISGGLFLIGVDNSILYTALPLLREQLAATETQALWIINAYPLLMAGLLLGTGTLGDKIGHRRMFLMGLSIFGIASLGAAFAPTAWALVAARAFLGIGAATMMPATLALIRITFEDERERNTAIGIWGSVSILGAAAGPIIGGALLEFFWWGSVFLINVPVAVIALIATLFVAPANIANPSKHWDFLSSFYALLTLAGLIITIKESVNTARHMPLLLGAVIMLIIGAVLFSSRQKKIEEPLLDLSLFRNRLFLGGVVAAGMAMFTVSGLEMTTSQRFQLSVGFTPLEAGLLMIPAALGSFPMSIIGGANLHRWGFKPLISGGFAATAVGIALCIWGATHTDGLPFFIAGLFFMGAGAGSVMSVSSTAIIGSAPVRKAGMASSIEEVSYEFGTLLSVAILGSLFPFFYSLHAPAEVADNFSAGVHHAIDGDAARASLDTAYINVLIIALVCAVAAALISSYLFRGNPKGANNAH

SEQ ID NO: 4 - protein, 494 aa, Artificial Sequence
  ATCC13869 NCgl2522_M2
MISETLQAQAPTKTQRWAFLAVISGGLFLIGVDNSILYTALPLLREQLAATETQALWIINAYPLLMAGLLLGTGTLGDKIGHRRMFLMGLSIFGIASLGAAFAPTAWALVAARAFLGIGAATMMPATLALIRITFEDERERNTAIGIWGSVSILGAAAGPIIGGALLEFFWWGSVFLINVPVAVIALIATLFVAPANIANPSKHWDFLSSFYALLTLAGLIVTIKESVNTARHLPLLVGAIILLIIGAVLFSSRQKKIEEPLLDLSLFRNRLFLGGVVAAGMAMFTVSGLEMTTSQRFQLSVGFTPLEAGLLMIPAALGSFPMSIIGGANLHRWGFKPLISGGFLATAVGIALCIWGATHTDGLPFFIAGLFFMGAGAGSVMSVSSTAIIGSAPVRKAGMASSIEEVSYEFGTLLSVAILGSLFPFFYSLHAPAEVADNFSAGVHHAIYGDAARASLDTAYINVLIIALVCAVAAALISSYLFRGNPKGANNAH

SEQ ID NO: 5 - protein, 494 aa, Artificial Sequence
  ATCC13032 NCgl2522_M3
MTSETLQAQAPTKTQRWAFLAVISGGLFLIGVDNSILYTALPLLREQLAATETQALWIINAYPLLMAGLLLGTGTLGDKIGHRRMFLMGLSIFGIASLGAAFAPTAWALVAARAFLGIGAATMMPATLALIRITFEDERERNTAIGIWGSVNILGAAAGPIIGGALLEFFWWGSVFLINVPVAVIALIATLFVAPANIANPSKHWDFLSSFYALLTLAGLIITIKESVNTARHMPLLLGAVIMLIIGAVLFSSRQKKIEEPLLDLSLFRNRLFLGGVVAAGMAMFTVSGLEMTTSQRFQLSVGFTPLEAGLLMIPAALGSFPMSIIGGANLHRWGFKPLISGGFAATAVGIALCIWGATHTDGLPFFIAGLFFMGAGAGSVMSVSSTAIIGSAPVRKAGMASSIEEVSYEFGTLLSVAILGSLFPFFYSLHAPAEVADNFSAGVHHAIDGDAARASLDTAYINVLIIALVCAVAAALISSYLFRGNPKGANNAH

SEQ ID NO: 6 - protein, 494 aa, Artificial Sequence
  ATCC13032 NCgl2522_M4
MTSETLQAQAPTKTQRWAFLAVISGGLFLIGVDNSILYTALPLLREQLAATETQALWIINAYPLLMAGLLLGTGTLGDKIGHRRMFLMGLSIFGIASLGAAFAPTAWALVAARAFLGIGAATMMPATLALIRITFEDERERNTAIGIWGSVHILGAAAGPIIGGALLEFFWWGSVFLINVPVAVIALIATLFVAPANIANPSKHWDFLSSFYALLTLAGLIITIKESVNTARHMPLLLGAVIMLIIGAVLFSSRQKKIEEPLLDLSLFRNRLFLGGVVAAGMAMFTVSGLEMTTSQRFQLSVGFTPLEAGLLMIPAALGSFPMSIIGGANLHRWGFKPLISGGFAATAVGIALCIWGATHTDGLPFFIAGLFFMGAGAGSVMSVSSTAIIGSAPVRKAGMASSIEEVSYEFGTLLSVAILGSLFPFFYSLHAPAEVADNFSAGVHHAIDGDAARASLDTAYINVLIIALVCAVAAALISSYLFRGNPKGANNAH

SEQ ID NO: 7 - protein, 494 aa, Artificial Sequence
  ATCC13032 NCgl2522_M5
MTSETLQAQAPTKTQRWAFLAVISGGLFLIGVDNSILYTALPLLREQLAATETQALWIINAYPLLMAGLLLGTGTLGDKIGHRRMFLMGLSIFGIASLGAAFAPTAWALVAARAFLGIGAATMMPATLALIRITFEDERERNTAIGIWGSVPILGAAAGPIIGGALLEFFWWGSVFLINVPVAVIALIATLFVAPANIANPSKHWDFLSSFYALLTLAGLIITIKESVNTARHMPLLLGAVIMLIIGAVLFSSRQKKIEEPLLDLSLFRNRLFLGGVVAAGMAMFTVSGLEMTTSQRFQLSVGFTPLEAGLLMIPAALGSFPMSIIGGANLHRWGFKPLISGGFAATAVGIALCIWGATHTDGLPFFIAGLFFMGAGAGSVMSVSSTAIIGSAPVRKAGMASSIEEVSYEFGTLLSVAILGSLFPFFYSLHAPAEVADNFSAGVHHAIDGDAARASLDTAYINVLIIALVCAVAAALISSYLFRGNPKGANNAH

SEQ ID NO: 8 - protein, 494 aa, Artificial Sequence
  ATCC13032 NCgl2522_M6
MTSETLQAQAPTKTQRWAFLAVISGGLFLIGVDNSILYTALPLLREQLAATETQALWIINAYPLLMAGLLLGTGTLGDKIGHRRMFLMGLSIFGIASLGAAFAPTAWALVAARAFLGIGAATMMPATLALIRITFEDERERNTAIGIWGSVKILGAAAGPIIGGALLEFFWWGSVFLINVPVAVIALIATLFVAPANIANPSKHWDFLSSFYALLTLAGLIITIKESVNTARHMPLLLGAVIMLIIGAVLFSSRQKKIEEPLLDLSLFRNRLFLGGVVAAGMAMFTVSGLEMTTSQRFQLSVGFTPLEAGLLMIPAALGSFPMSIIGGANLHRWGFKPLISGGFAATAVGIALCIWGATHTDGLPFFIAGLFFMGAGAGSVMSVSSTAIIGSAPVRKAGMASSIEEVSYEFGTLLSVAILGSLFPFFYSLHAPAEVADNFSAGVHHAIDGDAARASLDTAYINVLIIALVCAVAAALISSYLFRGNPKGANNAH

SEQ ID NO: 9 - protein, 494 aa, Artificial Sequence
  ATCC13032 NCgl2522_M7
MTSETLQAQAPTKTQRWAFLAVISGGLFLIGVDNSILYTALPLLREQLAATETQALWIINAYPLLMAGLLLGTGTLGDKIGHRRMFLMGLSIFGIASLGAAFAPTAWALVAARAFLGIGAATMMPATLALIRITFEDERERNTAIGIWGSVEILGAAAGPIIGGALLEFFWWGSVFLINVPVAVIALIATLFVAPANIANPSKHWDFLSSFYALLTLAGLIITIKESVNTARHMPLLLGAVIMLIIGAVLFSSRQKKIEEPLLDLSLFRNRLFLGGVVAAGMAMFTVSGLEMTTSQRFQLSVGFTPLEAGLLMIPAALGSFPMSIIGGANLHRWGFKPLISGGFAATAVGIALCIWGATHTDGLPFFIAGLFFMGAGAGSVMSVSSTAIIGSAPVRKAGMASSIEEVSYEFGTLLSVAILGSLFPFFYSLHAPAEVADNFSAGVHHAIDGDAARASLDTAYINVLIIALVCAVAAALISSYLFRGNPKGANNAH

SEQ ID NO: 10 - protein, 494 aa, Artificial Sequence
  ATCC13032 NCgl2522_M8
MTSETLQAQAPTKTQRWAFLAVISGGLFLIGVDNSILYTALPLLREQLAATETQALWIINAYPLLMAGLLLGTGTLGDKIGHRRMFLMGLSIFGIASLGAAFAPTAWALVAARAFLGIGAATMMPATLALIRITFEDERERNTAIGIWGSVCILGAAAGPIIGGALLEFFWWGSVFLINVPVAVIALIATLFVAPANIANPSKHWDFLSSFYALLTLAGLIITIKESVNTARHMPLLLGAVIMLIIGAVLFSSRQKKIEEPLLDLSLFRNRLFLGGVVAAGMAMFTVSGLEMTTSQRFQLSVGFTPLEAGLLMIPAALGSFPMSIIGGANLHRWGFKPLISGGFAATAVGIALCIWGATHTDGLPFFIAGLFFMGAGAGSVMSVSSTAIIGSAPVRKAGMASSIEEVSYEFGTLLSVAILGSLFPFFYSLHAPAEVADNFSAGVHHAIDGDAARASLDTAYINVLIIALVCAVAAALISSYLFRGNPKGANNAH

SEQ ID NO: 11 - protein, 494 aa, Artificial Sequence
  ATCC13032 NCgl2522_M9
MTSETLQAQAPTKTQRWAFLAVISGGLFLIGVDNSILYTALPLLREQLAATETQALWIINAYPLLMAGLLLGTGTLGDKIGHRRMFLMGLSIFGIASLGAAFAPTAWALVAARAFLGIGAATMMPATLALIRITFEDERERNTAIGIWGSVQILGAAAGPIIGGALLEFFWWGSVFLINVPVAVIALIATLFVAPANIANPSKHWDFLSSFYALLTLAGLIITIKESVNTARHMPLLLGAVIMLIIGAVLFSSRQKKIEEPLLDLSLFRNRLFLGGVVAAGMAMFTVSGLEMTTSQRFQLSVGFTPLEAGLLMIPAALGSFPMSIIGGANLHRWGFKPLISGGFAATAVGIALCIWGATHTDGLPFFIAGLFFMGAGAGSVMSVSSTAIIGSAPVRKAGMASSIEEVSYEFGTLLSVAILGSLFPFFYSLHAPAEVADNFSAGVHHAIDGDAARASLDTAYINVLIIALVCAVAAALISSYLFRGNPKGANNAH

SEQ ID NO: 12 - protein, 494 aa, Artificial Sequence
  ATCC13032 NCgl2522_M10
MTSETLQAQAPTKTQRWAFLAVISGGLFLIGVDNSILYTALPLLREQLAATETQALWIINAYPLLMAGLLLGTGTLGDKIGHRRMFLMGLSIFGIASLGAAFAPTAWALVAARAFLGIGAATMMPATLALIRITFEDERERNTAIGIWGSVMILGAAAGPIIGGALLEFFWWGSVFLINVPVAVIALIATLFVAPANIANPSKHWDFLSSFYALLTLAGLIITIKESVNTARHMPLLLGAVIMLIIGAVLFSSRQKKIEEPLLDLSLFRNRLFLGGVVAAGMAMFTVSGLEMTTSQRFQLSVGFTPLEAGLLMIPAALGSFPMSIIGGANLHRWGFKPLISGGFAATAVGIALCIWGATHTDGLPFFIAGLFFMGAGAGSVMSVSSTAIIGSAPVRKAGMASSIEEVSYEFGTLLSVAILGSLFPFFYSLHAPAEVADNFSAGVHHAIDGDAARASLDTAYINVLIIALVCAVAAALISSYLFRGNPKGANNAH

SEQ ID NO: 13 - protein, 494 aa, Artificial Sequence
  ATCC13869 NCgl2522_M11
MISETLQAQAPTKTQRWAFLAVISGGLFLIGVDNSILYTALPLLREQLAATETQALWIINAYPLLMAGLLLGTGTLGDKIGHRRMFLMGLSIFGIASLGAAFAPTAWALVAARAFLGIGAATMMPATLALIRITFEDERERNTAIGIWGSVNILGAAAGPIIGGALLEFFWWGSVFLINVPVAVIALIATLFVAPANIANPSKHWDFLSSFYALLTLAGLIVTIKESVNTARHLPLLVGAIILLIIGAVLFSSRQKKIEEPLLDLSLFRNRLFLGGVVAAGMAMFTVSGLEMTTSQRFQLSVGFTPLEAGLLMIPAALGSFPMSIIGGANLHRWGFKPLISGGFLATAVGIALCIWGATHTDGLPFFIAGLFFMGAGAGSVMSVSSTAIIGSAPVRKAGMASSIEEVSYEFGTLLSVAILGSLFPFFYSLHAPAEVADNFSAGVHHAIYGDAARASLDTAYINVLIIALVCAVAAALISSYLFRGNPKGANNAH

SEQ ID NO: 14 - protein, 494 aa, Artificial Sequence
  ATCC13869 NCgl2522_M12
MISETLQAQAPTKTQRWAFLAVISGGLFLIGVDNSILYTALPLLREQLAATETQALWIINAYPLLMAGLLLGTGTLGDKIGHRRMFLMGLSIFGIASLGAAFAPTAWALVAARAFLGIGAATMMPATLALIRITFEDERERNTAIGIWGSVHILGAAAGPIIGGALLEFFWWGSVFLINVPVAVIALIATLFVAPANIANPSKHWDFLSSFYALLTLAGLIVTIKESVNTARHLPLLVGAIILLIIGAVLFSSRQKKIEEPLLDLSLFRNRLFLGGVVAAGMAMFTVSGLEMTTSQRFQLSVGFTPLEAGLLMIPAALGSFPMSIIGGANLHRWGFKPLISGGFLATAVGIALCIWGATHTDGLPFFIAGLFFMGAGAGSVMSVSSTAIIGSAPVRKAGMASSIEEVSYEFGTLLSVAILGSLFPFFYSLHAPAEVADNFSAGVHHAIYGDAARASLDTAYINVLIIALVCAVAAALISSYLFRGNPKGANNAH

SEQ ID NO: 15 - protein, 494 aa, Artificial Sequence
  ATCC13869 NCgl2522_M13
MISETLQAQAPTKTQRWAFLAVISGGLFLIGVDNSILYTALPLLREQLAATETQALWIINAYPLLMAGLLLGTGTLGDKIGHRRMFLMGLSIFGIASLGAAFAPTAWALVAARAFLGIGAATMMPATLALIRITFEDERERNTAIGIWGSVPILGAAAGPIIGGALLEFFWWGSVFLINVPVAVIALIATLFVAPANIANPSKHWDFLSSFYALLTLAGLIVTIKESVNTARHLPLLVGAIILLIIGAVLFSSRQKKIEEPLLDLSLFRNRLFLGGVVAAGMAMFTVSGLEMTTSQRFQLSVGFTPLEAGLLMIPAALGSFPMSIIGGANLHRWGFKPLISGGFLATAVGIALCIWGATHTDGLPFFIAGLFFMGAGAGSVMSVSSTAIIGSAPVRKAGMASSIEEVSYEFGTLLSVAILGSLFPFFYSLHAPAEVADNFSAGVHHAIYGDAARASLDTAYINVLIIALVCAVAAALISSYLFRGNPKGANNAH

SEQ ID NO: 16 - protein, 494 aa, Artificial Sequence
  ATCC13869 NCgl2522_M14
MISETLQAQAPTKTQRWAFLAVISGGLFLIGVDNSILYTALPLLREQLAATETQALWIINAYPLLMAGLLLGTGTLGDKIGHRRMFLMGLSIFGIASLGAAFAPTAWALVAARAFLGIGAATMMPATLALIRITFEDERERNTAIGIWGSVKILGAAAGPIIGGALLEFFWWGSVFLINVPVAVIALIATLFVAPANIANPSKHWDFLSSFYALLTLAGLIVTIKESVNTARHLPLLVGAIILLIIGAVLFSSRQKKIEEPLLDLSLFRNRLFLGGVVAAGMAMFTVSGLEMTTSQRFQLSVGFTPLEAGLLMIPAALGSFPMSIIGGANLHRWGFKPLISGGFLATAVGIALCIWGATHTDGLPFFIAGLFFMGAGAGSVMSVSSTAIIGSAPVRKAGMASSIEEVSYEFGTLLSVAILGSLFPFFYSLHAPAEVADNFSAGVHHAIYGDAARASLDTAYINVLIIALVCAVAAALISSYLFRGNPKGANNAH

SEQ ID NO: 17 - protein, 494 aa, Artificial Sequence
  ATCC13869 NCgl2522_M15
MISETLQAQAPTKTQRWAFLAVISGGLFLIGVDNSILYTALPLLREQLAATETQALWIINAYPLLMAGLLLGTGTLGDKIGHRRMFLMGLSIFGIASLGAAFAPTAWALVAARAFLGIGAATMMPATLALIRITFEDERERNTAIGIWGSVEILGAAAGPIIGGALLEFFWWGSVFLINVPVAVIALIATLFVAPANIANPSKHWDFLSSFYALLTLAGLIVTIKESVNTARHLPLLVGAIILLIIGAVLFSSRQKKIEEPLLDLSLFRNRLFLGGVVAAGMAMFTVSGLEMTTSQRFQLSVGFTPLEAGLLMIPAALGSFPMSIIGGANLHRWGFKPLISGGFLATAVGIALCIWGATHTDGLPFFIAGLFFMGAGAGSVMSVSSTAIIGSAPVRKAGMASSIEEVSYEFGTLLSVAILGSLFPFFYSLHAPAEVADNFSAGVHHAIYGDAARASLDTAYINVLIIALVCAVAAALISSYLFRGNPKGANNAH

SEQ ID NO: 18 - protein, 494 aa, Artificial Sequence
  ATCC13869 NCgl2522_M16
MISETLQAQAPTKTQRWAFLAVISGGLFLIGVDNSILYTALPLLREQLAATETQALWIINAYPLLMAGLLLGTGTLGDKIGHRRMFLMGLSIFGIASLGAAFAPTAWALVAARAFLGIGAATMMPATLALIRITFEDERERNTAIGIWGSVCILGAAAGPIIGGALLEFFWWGSVFLINVPVAVIALIATLFVAPANIANPSKHWDFLSSFYALLTLAGLIVTIKESVNTARHLPLLVGAIILLIIGAVLFSSRQKKIEEPLLDLSLFRNRLFLGGVVAAGMAMFTVSGLEMTTSQRFQLSVGFTPLEAGLLMIPAALGSFPMSIIGGANLHRWGFKPLISGGFLATAVGIALCIWGATHTDGLPFFIAGLFFMGAGAGSVMSVSSTAIIGSAPVRKAGMASSIEEVSYEFGTLLSVAILGSLFPFFYSLHAPAEVADNFSAGVHHAIYGDAARASLDTAYINVLIIALVCAVAAALISSYLFRGNPKGANNAH

SEQ ID NO: 19 - protein, 494 aa, Artificial Sequence
  ATCC13869 NCgl2522_M17
MISETLQAQAPTKTQRWAFLAVISGGLFLIGVDNSILYTALPLLREQLAATETQALWIINAYPLLMAGLLLGTGTLGDKIGHRRMFLMGLSIFGIASLGAAFAPTAWALVAARAFLGIGAATMMPATLALIRITFEDERERNTAIGIWGSVQILGAAAGPIIGGALLEFFWWGSVFLINVPVAVIALIATLFVAPANIANPSKHWDFLSSFYALLTLAGLIVTIKESVNTARHLPLLVGAIILLIIGAVLFSSRQKKIEEPLLDLSLFRNRLFLGGVVAAGMAMFTVSGLEMTTSQRFQLSVGFTPLEAGLLMIPAALGSFPMSIIGGANLHRWGFKPLISGGFLATAVGIALCIWGATHTDGLPFFIAGLFFMGAGAGSVMSVSSTAIIGSAPVRKAGMASSIEEVSYEFGTLLSVAILGSLFPFFYSLHAPAEVADNFSAGVHHAIYGDAARASLDTAYINVLIIALVCAVAAALISSYLFRGNPKGANNAH

SEQ ID NO: 20 - protein, 494 aa, Artificial Sequence
  ATCC13869 NCgl2522_M18
MISETLQAQAPTKTQRWAFLAVISGGLFLIGVDNSILYTALPLLREQLAATETQALWIINAYPLLMAGLLLGTGTLGDKIGHRRMFLMGLSIFGIASLGAAFAPTAWALVAARAFLGIGAATMMPATLALIRITFEDERERNTAIGIWGSVMILGAAAGPIIGGALLEFFWWGSVFLINVPVAVIALIATLFVAPANIANPSKHWDFLSSFYALLTLAGLIVTIKESVNTARHLPLLVGAIILLIIGAVLFSSRQKKIEEPLLDLSLFRNRLFLGGVVAAGMAMFTVSGLEMTTSQRFQLSVGFTPLEAGLLMIPAALGSFPMSIIGGANLHRWGFKPLISGGFLATAVGIALCIWGATHTDGLPFFIAGLFFMGAGAGSVMSVSSTAIIGSAPVRKAGMASSIEEVSYEFGTLLSVAILGSLFPFFYSLHAPAEVADNFSAGVHHAIYGDAARASLDTAYINVLIIALVCAVAAALISSYLFRGNPKGANNAH

SEQ ID NO: 21 - DNA, 36 bp, Artificial Sequence
  13032-putE-EF-FX
ccggggatcctctagaacttcagaaaccttacaggc

SEQ ID NO: 22 - DNA, 36 bp, Artificial Sequence
  13032-putE-EF-RX
gcaggtcgactctagactagtgcgcattattggctc

SEQ ID NO: 23 - DNA, 27 bp, Artificial Sequence
  SM_putE_A152-F
tggggttccgtgnnkattcttggcgct

SEQ ID NO: 24 - DNA, 27 bp, Artificial Sequence
  SM_putE_A152-R
agcgccaagaatmnncacggaacccca

SEQ ID NO: 25 - DNA, 34 bp, Artificial Sequence
  pDC-putE-up-FX
ccggggatcctctagagtggtctctttctgatcg

SEQ ID NO: 26 - DNA, 34 bp, Artificial Sequence
  pDC-putE-down-RX
gcaggtcgactctagagcaattccttgtcccagt

SEQ ID NO: 27 - DNA, 23 bp, Artificial Sequence
  13032-putE-A152S-F
gggttccgtgtccattcttggcg

SEQ ID NO: 28 - DNA, 23 bp, Artificial Sequence
  13032-putE-A152S-R
cgccaagaatggacacggaaccc

SEQ ID NO: 29 - DNA, 23 bp, Artificial Sequence
  13032-putE-A152N-F
gggttccgtgaatattcttggcg

SEQ ID NO: 30 - DNA, 23 bp, Artificial Sequence
  13032-putE-A152N-R
cgccaagaatattcacggaaccc

SEQ ID NO: 31 - DNA, 23 bp, Artificial Sequence
  13032-putE-A152H-F
gggttccgtgcatattcttggcg

SEQ ID NO: 32 - DNA, 23 bp, Artificial Sequence
  13032-putE-A152H-R
cgccaagaatatgcacggaaccc

SEQ ID NO: 33 - DNA, 23 bp, Artificial Sequence
  13032-putE-A152P-F
gggttccgtgcctattcttggcg

SEQ ID NO: 34 - DNA, 23 bp, Artificial Sequence
  13032-putE-A152P-R
cgccaagaataggcacggaaccc

SEQ ID NO: 35 - DNA, 23 bp, Artificial Sequence
  13032-putE-A152K-F
gggttccgtgaagattcttggcg

SEQ ID NO: 36 - DNA, 23 bp, Artificial Sequence
  13032-putE-A152K-R
cgccaagaatcttcacggaaccc

SEQ ID NO: 37 - DNA, 23 bp, Artificial Sequence
  13032-putE-A152E-F
gggttccgtggagattcttggcg

SEQ ID NO: 38 - DNA, 23 bp, Artificial Sequence
  13032-putE-A152E-R
cgccaagaatctccacggaaccc

SEQ ID NO: 39 - DNA, 23 bp, Artificial Sequence
  13032-putE-A152C-F
gggttccgtgtgtattcttggcg

SEQ ID NO: 40 - DNA, 23 bp, Artificial Sequence
  13032-putE-A152C-R
cgccaagaatacacacggaaccc

SEQ ID NO: 41 - DNA, 23 bp, Artificial Sequence
  13032-putE-A152Q-F
gggttccgtgcagattcttggcg

SEQ ID NO: 42 - DNA, 23 bp, Artificial Sequence
  13032-putE-A152Q-R
cgccaagaatctgcacggaaccc

SEQ ID NO: 43 - DNA, 23 bp, Artificial Sequence
  13032-putE-A152M-F
gggttccgtgatgattcttggcg

SEQ ID NO: 44 - DNA, 23 bp, Artificial Sequence
  13032-putE-A152M-R
cgccaagaatcatcacggaaccc

SEQ ID NO: 45 - DNA, 23 bp, Artificial Sequence
  13869-putE-A152S-F
gggttctgtgtccattcttggcg

SEQ ID NO: 46 - DNA, 23 bp, Artificial Sequence
  13869-putE-A152S-R
cgccaagaatggacacagaaccc

SEQ ID NO: 47 - DNA, 23 bp, Artificial Sequence
  13869-putE-A152N-F
gggttctgtgaatattcttggcg

SEQ ID NO: 48 - DNA, 23 bp, Artificial Sequence
  13869-putE-A152N-R
cgccaagaatattcacagaaccc

SEQ ID NO: 49 - DNA, 23 bp, Artificial Sequence
  13869-putE-A152H-F
gggttctgtgcatattcttggcg

SEQ ID NO: 50 - DNA, 23 bp, Artificial Sequence
  13869-putE-A152H-R
cgccaagaatatgcacagaaccc

SEQ ID NO: 51 - DNA, 23 bp, Artificial Sequence
  13869-putE-A152P-F
gggttctgtgcctattcttggcg

SEQ ID NO: 52 - DNA, 23 bp, Artificial Sequence
  13869-putE-A152P-R
cgccaagaataggcacagaaccc

SEQ ID NO: 53 - DNA, 23 bp, Artificial Sequence
  13869-putE-A152K-F
gggttctgtgaagattcttggcg

SEQ ID NO: 54 - DNA, 23 bp, Artificial Sequence
  13869-putE-A152K-R
cgccaagaatcttcacagaaccc

SEQ ID NO: 55 - DNA, 23 bp, Artificial Sequence
  13869-putE-A152E-F
gggttctgtggagattcttggcg

SEQ ID NO: 56 - DNA, 23 bp, Artificial Sequence
  13869-putE-A152E-R
cgccaagaatctccacagaaccc

SEQ ID NO: 57 - DNA, 23 bp, Artificial Sequence
  13869-putE-A152C-F
gggttctgtgtgtattcttggcg

SEQ ID NO: 58 - DNA, 23 bp, Artificial Sequence
  13869-putE-A152C-R
cgccaagaatacacacagaaccc

SEQ ID NO: 59 - DNA, 23 bp, Artificial Sequence
  13869-putE-A152Q-F
gggttctgtgcagattcttggcg

SEQ ID NO: 60 - DNA, 23 bp, Artificial Sequence
  13869-putE-A152Q-R
cgccaagaatctgcacagaaccc

SEQ ID NO: 61 - DNA, 23 bp, Artificial Sequence
  13869-putE-A152M-F
gggttctgtgatgattcttggcg

SEQ ID NO: 62 - DNA, 23 bp, Artificial Sequence
  13869-putE-A152M-R
cgccaagaatcatcacagaaccc

SEQ ID NO: 63 - DNA, 37 bp, Artificial Sequence
  NCgl2522-L5
tgcaggtcgactctagagttctgcgtagctgtgtgcc

SEQ ID NO: 64 - DNA, 31 bp, Artificial Sequence
  NCgl2522-L3
gatgtttctggatcgtaactgtaacgaatgg

SEQ ID NO: 65 - DNA, 24 bp, Artificial Sequence
  CJ7-F
agaaacatcccagcgctactaata

SEQ ID NO: 66 - DNA, 23 bp, Artificial Sequence
  CJ7-R
agtgtttcctttcgttgggtacg

SEQ ID NO: 67 - DNA, 41 bp, Artificial Sequence
  NCgl2522-R5
caacgaaaggaaacactatgatttcagaaactttgcaggcg

SEQ ID NO: 68 - DNA, 40 bp, Artificial Sequence
  NCgl2522-R3
tcggtacccggggatcccacaaaaagcgtagcgatcaacg